European Patent Application EP 4 772 621 A1, published July 8, 2026. Title: 耐盐性提高的全能核酸酶变体及应用. Applicant: 北京百普赛斯生物科技股份有限公司. Application CN. The sequence listing filed with the application follows.

SEQUENCE LISTING (16 sequences)

SEQ ID NO: 1 - protein, 266 aa, Serratia marcescens
MRFNNKMLALAALLFAAQASADTLESIDNCAVGCPTGGSSNVSIVRHAYTLNNNSTTKFANWVAYHITKDTPASGKTRNWKTDPALNPADTLAPADYTGANAALKVDRGHQAPLASLAGVSDWESLNYLSNITPQKSDLNQGAWARLEDQERKLIDRADISSVYTVTGPLYERDMGKLPGTQKAHTIPSAYWKVIFINNSPAVNHYAAFLFDQNTPKGADFCQFRVTVDEIEKRTGLIIWAGLPDDVQASLKSKPGVLPELMGCKN

SEQ ID NO: 2 - protein, 266 aa, synthetic construct
MRFNNKMLALAALLFAAQASADTLESIDNCAVGCPTGGSSNVSIVRHAYTLNNNSDTKFANWVAYHITKDTPASGKTRNWKTDPALNPADTLAPADYTGANAALKVDRGHQAPLASLAGVSDWESLNYLSNITPQKSDLNQGAWARLEDQERKLIDRADISSVYTVTGPLYERDMGKLPGTQKAHTIPSAYWKVIFINNSPAVNHYAAFLFDQNTPKGADFCQFRVTVDEIEKRTGLIIWAGLPDDVQASLKSKPGVLPELMGCKN

SEQ ID NO: 3 - protein, 266 aa, synthetic construct
MRFNNKMLALAALLFAAQASADTLESIDNCAVGCPTGGSSNVSIVRHAYTLNNNSTTKFANWVAYHITKDTPASGKTRNWKTDPALNPADTLAPADYKGANAALKVDRGHQAPLASLAGVSDWESLNYLSNITPQKSDLNQGAWARLEDQERKLIDRADISSVYTVTGPLYERDMGKLPGTQKAHTIPSAYWKVIFINNSPAVNHYAAFLFDQNTPKGADFCQFRVTVDEIEKRTGLIIWAGLPDDVQASLKSKPGVLPELMGCKN

SEQ ID NO: 4 - protein, 266 aa, synthetic construct
MRFNNKMLALAALLFAAQASADTLESIDNCAVGCPTGGSSNVSIVRHAYTLNNNSTTKFANWVAYHITKDTPASGKTRNWKTDPALNPADTLAPADYTGAHAALKVDRGHQAPLASLAGVSDWESLNYLSNITPQKSDLNQGAWARLEDQERKLIDRADISSVYTVTGPLYERDMGKLPGTQKAHTIPSAYWKVIFINNSPAVNHYAAFLFDQNTPKGADFCQFRVTVDEIEKRTGLIIWAGLPDDVQASLKSKPGVLPELMGCKN

SEQ ID NO: 5 - protein, 266 aa, synthetic construct
MRFNNKMLALAALLFAAQASADTLESIDNCAVGCPTGGSSNVSIVRHAYTLNNNSTTKFANWVAYHITKDTPASGKTRNWKTDPALNPADTLAPADYTGANAALKVDRGHQAPLASLAGVSDWESLNYLSNITPQKSDLNQGAWARLEDQERKLIDRADISSVYTVTGPLYERDMGKLPGTQKAHTIPSAYWKVIFINNSPAVNHYAAFLFDQNTPKGADFCQFRVTVDEIEKRTGLIIWADLPDDVQASLKSKPGVLPELMGCKN

SEQ ID NO: 6 - protein, 266 aa, synthetic construct
MRFNNKMLALAALLFAAQASADTLESIDNCAVGCPTGGSSNVSIVRHAYTLNNNSDTKFANWVAYHITKDTPASGKTRNWKTDPALNPADTLAPADYKGANAALKVDRGHQAPLASLAGVSDWESLNYLSNITPQKSDLNQGAWARLEDQERKLIDRADISSVYTVTGPLYERDMGKLPGTQKAHTIPSAYWKVIFINNSPAVNHYAAFLFDQNTPKGADFCQFRVTVDEIEKRTGLIIWAGLPDDVQASLKSKPGVLPELMGCKN

SEQ ID NO: 7 - protein, 266 aa, synthetic construct
MRFNNKMLALAALLFAAQASADTLESIDNCAVGCPTGGSSNVSIVRHAYTLNNNSDTKFANWVAYHITKDTPASGKTRNWKTDPALNPADTLAPADYTGANAALKVDRGHQAPLASLAGVSDWESLNYLSNITPQKSDLNQGAWARLEDQERKLIDRADISSVYTVTGPLYERDMGKLPGTQKAHTIPSAYWKVIFINNSPAVNHYAAFLFDQNTPKGADFCQFRVTVDEIEKRTGLIIWADLPDDVQASLKSKPGVLPELMGCKN

SEQ ID NO: 8 - protein, 266 aa, synthetic construct
MRFNNKMLALAALLFAAQASADTLESIDNCAVGCPTGGSSNVSIVRHAYTLNNNSDTKFANWVAYHITKDTPASGKTRNWKTDPALNPADTLAPADYTGAHAALKVDRGHQAPLASLAGVSDWESLNYLSNITPQKSDLNQGAWARLEDQERKLIDRADISSVYTVTGPLYERDMGKLPGTQKAHTIPSAYWKVIFINNSPAVNHYAAFLFDQNTPKGADFCQFRVTVDEIEKRTGLIIWAGLPDDVQASLKSKPGVLPELMGCKN

SEQ ID NO: 9 - protein, 266 aa, synthetic construct
MRFNNKMLALAALLFAAQASADTLESIDNCAVGCPTGGSSNVSIVRHAYTLNNNSTTKFANWVAYHITKDTPASGKTRNWKTDPALNPADTLAPADYKGANAALKVDRGHQAPLASLAGVSDWESLNYLSNITPQKSDLNQGAWARLEDQERKLIDRADISSVYTVTGPLYERDMGKLPGTQKAHTIPSAYWKVIFINNSPAVNHYAAFLFDQNTPKGADFCQFRVTVDEIEKRTGLIIWADLPDDVQASLKSKPGVLPELMGCKN

SEQ ID NO: 10 - protein, 266 aa, synthetic construct
MRFNNKMLALAALLFAAQASADTLESIDNCAVGCPTGGSSNVSIVRHAYTLNNNSTTKFANWVAYHITKDTPASGKTRNWKTDPALNPADTLAPADYKGAHAALKVDRGHQAPLASLAGVSDWESLNYLSNITPQKSDLNQGAWARLEDQERKLIDRADISSVYTVTGPLYERDMGKLPGTQKAHTIPSAYWKVIFINNSPAVNHYAAFLFDQNTPKGADFCQFRVTVDEIEKRTGLIIWAGLPDDVQASLKSKPGVLPELMGCKN

SEQ ID NO: 11 - protein, 266 aa, synthetic construct
MRFNNKMLALAALLFAAQASADTLESIDNCAVGCPTGGSSNVSIVRHAYTLNNNSTTKFANWVAYHITKDTPASGKTRNWKTDPALNPADTLAPADYTGAHAALKVDRGHQAPLASLAGVSDWESLNYLSNITPQKSDLNQGAWARLEDQERKLIDRADISSVYTVTGPLYERDMGKLPGTQKAHTIPSAYWKVIFINNSPAVNHYAAFLFDQNTPKGADFCQFRVTVDEIEKRTGLIIWADLPDDVQASLKSKPGVLPELMGCKN

SEQ ID NO: 12 - protein, 266 aa, synthetic construct
MRFNNKMLALAALLFAAQASADTLESIDNCAVGCPTGGSSNVSIVRHAYTLNNNSDTKFANWVAYHITKDTPASGKTRNWKTDPALNPADTLAPADYKGAHAALKVDRGHQAPLASLAGVSDWESLNYLSNITPQKSDLNQGAWARLEDQERKLIDRADISSVYTVTGPLYERDMGKLPGTQKAHTIPSAYWKVIFINNSPAVNHYAAFLFDQNTPKGADFCQFRVTVDEIEKRTGLIIWAGLPDDVQASLKSKPGVLPELMGCKN

SEQ ID NO: 13 - protein, 266 aa, synthetic construct
MRFNNKMLALAALLFAAQASADTLESIDNCAVGCPTGGSSNVSIVRHAYTLNNNSDTKFANWVAYHITKDTPASGKTRNWKTDPALNPADTLAPADYKGANAALKVDRGHQAPLASLAGVSDWESLNYLSNITPQKSDLNQGAWARLEDQERKLIDRADISSVYTVTGPLYERDMGKLPGTQKAHTIPSAYWKVIFINNSPAVNHYAAFLFDQNTPKGADFCQFRVTVDEIEKRTGLIIWADLPDDVQASLKSKPGVLPELMGCKN

SEQ ID NO: 14 - protein, 266 aa, synthetic construct
MRFNNKMLALAALLFAAQASADTLESIDNCAVGCPTGGSSNVSIVRHAYTLNNNSTTKFANWVAYHITKDTPASGKTRNWKTDPALNPADTLAPADYKGAHAALKVDRGHQAPLASLAGVSDWESLNYLSNITPQKSDLNQGAWARLEDQERKLIDRADISSVYTVTGPLYERDMGKLPGTQKAHTIPSAYWKVIFINNSPAVNHYAAFLFDQNTPKGADFCQFRVTVDEIEKRTGLIIWADLPDDVQASLKSKPGVLPELMGCKN

SEQ ID NO: 15 - protein, 266 aa, synthetic construct
MRFNNKMLALAALLFAAQASADTLESIDNCAVGCPTGGSSNVSIVRHAYTLNNNSDTKFANWVAYHITKDTPASGKTRNWKTDPALNPADTLAPADYTGAHAALKVDRGHQAPLASLAGVSDWESLNYLSNITPQKSDLNQGAWARLEDQERKLIDRADISSVYTVTGPLYERDMGKLPGTQKAHTIPSAYWKVIFINNSPAVNHYAAFLFDQNTPKGADFCQFRVTVDEIEKRTGLIIWADLPDDVQASLKSKPGVLPELMGCKN

SEQ ID NO: 16 - protein, 266 aa, synthetic construct
MRFNNKMLALAALLFAAQASADTLESIDNCAVGCPTGGSSNVSIVRHAYTLNNNSDTKFANWVAYHITKDTPASGKTRNWKTDPALNPADTLAPADYKGAHAALKVDRGHQAPLASLAGVSDWESLNYLSNITPQKSDLNQGAWARLEDQERKLIDRADISSVYTVTGPLYERDMGKLPGTQKAHTIPSAYWKVIFINNSPAVNHYAAFLFDQNTPKGADFCQFRVTVDEIEKRTGLIIWADLPDDVQASLKSKPGVLPELMGCKN